European Patent Specification EP 3 555 127 B1, published December 18, 2024. Title: Agents, uses and methods. Applicant: Lundbeck A/S. The sequence listing filed with the application follows.

SEQUENCE LISTING (48 sequences)

SEQ ID NO: 1 - protein, 140 aa, Human alpha-synuclein
MDVFMKGLSKAKEGVVAAAEKTKQGVAEAAGKTKEGVLYVGSKTKEGVVHGVATVAEKTKEQVTNVGGAVVTGVTAVAQKTVEGAGSIAAATGFVKKDQLGKNEEGAPQEGILEDMPVDPDNEAYEMPSEEGYQDYEPEA

SEQ ID NO: 2 - protein, 15 aa, artificial
  Epitope 126-140
EMPSEEGYQDYEPEA

SEQ ID NO: 3 - protein, 10 aa, artificial
  CDR1 VL
SASSSVSYMH

SEQ ID NO: 4 - protein, 7 aa, artificial
  CDR2 VL
DTSKLAS

SEQ ID NO: 5 - protein, 9 aa, artificial
  CDR3 VL
QQWSSNPPT

SEQ ID NO: 6 - protein, 5 aa, artificial
  CDR1 VH
SYWMH

SEQ ID NO: 7 - protein, 17 aa, artificial
  CDR2 VH
RIDPNSGTTKYNVNFKT

SEQ ID NO: 8 - protein, 12 aa, artificial
  CDR3 VH
LGHYGNLYAMDY

SEQ ID NO: 9 - protein, 10 aa, artificial
  CDR1 VL 7C4
SASSSVSFMH

SEQ ID NO: 10 - protein, 10 aa, artificial
  CDR1 VL 7A10/8D9
SASSSVSYIH

SEQ ID NO: 11 - protein, 9 aa, artificial
  CDR3 VL L3
QQWTSNPPF

SEQ ID NO: 12 - protein, 5 aa, artificial
  CDR1 VH 7C4
RYWMH

SEQ ID NO: 13 - protein, 17 aa, artificial
  CDR2 VH 5A1
RVDPNSGTTKYNVNFKT

SEQ ID NO: 14 - protein, 17 aa, artificial
  CDR2 VH 9G11
RIDPNSGTTKYNVHFKT

SEQ ID NO: 15 - protein, 17 aa, artificial
  CDR2 VH 9C12
RIDPNSGTTKYNVNIKT

SEQ ID NO: 16 - protein, 12 aa, artificial
  CDR3 VH 5A1
LGHYGNLNAMDY

SEQ ID NO: 17 - protein, 12 aa, Artificial
  CDR3 VH 9D7
LGHYSKVLAMDY

SEQ ID NO: 18 - protein, 12 aa, artificial
  CDR3 VH 7A10/8D9
LGHYGNLYAKDY

SEQ ID NO: 19 - protein, 106 aa, artificial
  m2E6 VL
QIVLTQSPAIMSASPGEKVTMTCSASSSVSYMHWYQQKSGTSPKRWIYDTSKLASGVPTRFSGSGSGTSYSLTISSMDTEDAATYYCQQWSSNPPTFGAGTKLELK

SEQ ID NO: 20 - protein, 118 aa, artificial
  m2E6 VH
QVQLQQPGAELVKPGASVKLSCTASGYTFTSYWMHWMKQRPGRGLEWIGRIDPNSGTTKYNVNFKTKATLTVDKPSSTAYMHLSSLTSEDSAVYYCARLGHYGNLYAMDYWGQGTSVT

SEQ ID NO: 21 - protein, 106 aa, artificial; identical to SEQ ID NO: 19
  ch2E6 VL

SEQ ID NO: 22 - protein, 118 aa, artificial; identical to SEQ ID NO: 20
  ch2E6 VH

SEQ ID NO: 23 - protein, 107 aa, artificial
  2E6-HLD1 VL
EIVLTQSPATLSLSPGERATLSCSASSSVSYMHWYQQKPGQAPRRWIYDTSKLASGVPARFSGSGSGTDYTLTISSLEPEDFAVYYCQQWSSNPPTFGQGTKLEIKR

SEQ ID NO: 24 - protein, 118 aa, artificial
  2E6-HLD1 VH
QVQLVQSGAEVKKPGASVKVSCKASGYTFTSYWMHWMRQAPGQGLEWIGRIDPNSGTTKYNVNFKTRATLTVDKSTSTAYMELSSLRSEDTAVYYCARLGHYGNLYAMDYWGQGTLVT

SEQ ID NO: 25 - protein, 107 aa, artificial; identical to SEQ ID NO: 23
  2E6-HLD2 VL

SEQ ID NO: 26 - protein, 118 aa, Artificial
  2E6-HLD2 VH
QVQLVQSGAEVKKPGASVKVSCKASGYTFTSYWMHWVRQAPGQGLEWIGRIDPNSGTTKYNVNFKTRATLTVDKSTSTAYMELSSLRSEDTAVYYCARLGHYGNLYAMDYWGQGTLVT

SEQ ID NO: 27 - protein, 107 aa, artificial
  2E6-HLD 3 VL
EIVLTQSPATLSLSPGERATLSCSASSSVSYMHWYQQKPGQAPRRWIYDTSKLASGVPARFSGSGSGTDYTLTISSLEPEDFAVYYCQQWTSNPPNFGQGTKLEIKR

SEQ ID NO: 28 - protein, 118 aa, artificial
  2E6-HLD 3  VH
QVQLVQSGAEVKKPGASVKVSCKASGYTFTSYWMHWMRQAPGQGLEWIGRIDPNSGTTKYNVNFKTRVTLTVDKSTSTAYMELSSLRSEDTAVYYCARLGHYGNLYAMDYWGQGTLVT

SEQ ID NO: 29 - protein, 106 aa, artificial
  5A1 VL
EIVLTQSPATLSLSPGERATLSCSASSSVSYMHWYQQKPGQAPRRWIYDTSKLASGVPARFSGSGSGTDYTLTISRLEPEDFAVYYCQQWSSNPPTFGQGTKLEIK

SEQ ID NO: 30 - protein, 118 aa, artificial
  5A1 VH
QVQLVQSGAEVKKQGASVKVSCKASGYTFTSYWMHYMRQAPGQGLEWIGRVDPNSGTTKYNVNFKTRATLTVDKTTSTAYMELSSLRSEDTAVYYCARLGHYGNLNAMDYWGQGTLVT

SEQ ID NO: 31 - protein, 106 aa, artificial
  9D7 VL
EIVLTQSPATLSLSPGERATLSCSASSSVSYMHWYQQKPGQAPRRWIYDTSKLASGVPARFSGSGSGTDYTLTISSLEPEDFAVYYCQQWSSNPPTFGQGTKLEIK

SEQ ID NO: 32 - protein, 118 aa, artificial
  9D7 VH
QVQLVQSGAEVKKPGASVKVSCKASGYTFTSYWMHWMRQAPGQGLEWIGRIDPNSGTTKYNVNFKTRATLTVDKSTSTAYMELSSLRSEDTAVYYCARLGHYSKVLAMDYWGQGTLVT

SEQ ID NO: 33 - protein, 106 aa, artificial
  9G11 VL
EIVLTQSPATLSLSPGERATLSCSASSSVSYMHWYQQKQGQAPRRWIYDTSKLASGVPARFSGSGSGTDYTLTISSLEPEDFAVYYCQQWSSNPPTFGQGTKLEIK

SEQ ID NO: 34 - protein, 118 aa, artificial
  9G11 VH
QVQLVQSGAEVKKPGASVKVSCKASGYTFTSYWMHWMRQAPGQGLEWIGRIDPNSGTTKYNVHFKTRATLTVDKSTSTAYMELSSLRSEDTAVYYCARLGHYGNLYATDYWGQGTLVT

SEQ ID NO: 35 - protein, 106 aa, artificial
  7C4 VL
EIVLTQSPATLSLSPGERATLSCSASSSVSFMHWYQQKPGQAPRRWIYDTSKLASGVPARFSGSGSGTDYTLTISSLEPEDFAVYYCQQWSSNPPTFGQGTKLEIK

SEQ ID NO: 36 - protein, 118 aa, artificial
  7C4 VH
QVQLVQSGAEVKKPGASVKVSCKASGYTFTRYWMHWMRQAPGQGPEWIGRIDPNSGTTKYNVNFKTRATLTVDKSTSTAYMELSSLRSEDTAVYYCARLGHYGNLYAMDYWGQGTLVT

SEQ ID NO: 37 - protein, 106 aa, artificial; identical to SEQ ID NO: 31
  L3 VL

SEQ ID NO: 38 - protein, 118 aa, artificial
  L3 VH
QVQLVQQGAEVKKPGASVKVSCKASGYTFTSYWMHWMRQAPGQGLEWIGRIDPNSGTTKYNVNFKTRATLTVDKSTSTAYMELSSLRSEDTAVYYCARLGHYGNLYAMDYWGQGTLVT

SEQ ID NO: 39 - protein, 106 aa, artificial
  7A10 VL
EIVLTQSPATLSLSPGERATLSCSASSSVSYIHWYQQKPGQAPRRWIYDTSKLASGVPARFSGSGSGTDYTLTISSLEPEDFAVYYCQQWTSNPPNFGQGTKLEIK

SEQ ID NO: 40 - protein, 118 aa, artificial
  7A10 VH
QVQLVQSGAEVKKPGASVKVSCKASGYTFTSYWMHWMRQAPGQGLEWIGRIDPNSGTTKYNVNFKTRATLTVDKSTSTAYMELSSLRSEDTAVYYCARLGHYGNLYAKDYWGQGTLVT

SEQ ID NO: 41 - protein, 106 aa, artificial
  8D9 VL
EIVLTQSPATLSLSPGERATLSCSASSSVSYIHWYQQKPGQAPRRWIYDTSKLASGVPARFSGSGSGTDYTLTISSLEPEDFAVYYCQQWSSNPPTFGQGTKLEIK

SEQ ID NO: 42 - protein, 118 aa, artificial; identical to SEQ ID NO: 40
  8D9 VH

SEQ ID NO: 43 - protein, 106 aa, artificial
  9C12 VL
EIVLTQSPATLSLSPGERATLSCSASSSVSYMHWYQQKPGQAPRRLIYDTSKLASGVPARFSGSGSGTDYTLTISSLEPEDFAVYYCQQWSSNPPTFGQGTKLEIK

SEQ ID NO: 44 - protein, 118 aa, artificial
  9C12 VH
QVQLVQSGAEVKKPGASVKVSCKASGYTFTSYWMHWMRQAPGQGLEWIGRIDPNSGTTKYNVNIKTRATLTVDKSTSTAYMELSSLRSEDTAVYYCARLGHYGNLYAMDYWGQGTLVT

SEQ ID NO: 45 - protein, 106 aa, artificial; identical to SEQ ID NO: 43
  6B6 VL

SEQ ID NO: 46 - protein, 118 aa, artificial; identical to SEQ ID NO: 24
  6B6 VH

SEQ ID NO: 47 - protein, 446 aa, Artificial
  9E4 LC
EVQLVESGGGLVQPGGSLRLSCAASGFTFSNYGMSWVRQAPGKGLEWVASISSGGGSTYYPDNVKGRFTISRDNAKNSLYLQMNSLRAEDTAVYYCARGGAGIDYWGQGTLVTVSSASTKGPSVFPLAPSSKSTSGGTAALGCLVKDYFPEPVTVSWNSGALTSGVHTFPAVLQSSGLYSLSSVVTVPSSSLGTQTYICNVNHKPSNTKVDKRVEPKSCDKTHTCPPCPAPELLGGPSVFLFPPKPKDTLMISRTPEVTCVVVDVSHEDPEVKFNWYVDGVEVHNAKTKPREEQYNSTYRVVSVLTVLHQDWLNGKEYKCKVSNKALPAPIEKTISKAKGQPREPQVYTLPPSREEMTKNQVSLTCLVKGFYPSDIAVEWESNGQPENNYKTTPPVLDSDGSFFLYSKLTVDKSRWQQGNVFSCSVMHEALHNHYTQKSLSLSPGK

SEQ ID NO: 48 - protein, 220 aa, Artificial
  9E4 HC
DIQMTQSPSSLSASVGDRVTITCKSIQTLLYSSNQKNYLAWFQQKPGKAPKLLIYWASIRKSGVPSRFSGSGSGTDFTLTISSLQPEDLATYYCQQYYSYPLTFGGGTKLEIKRTVAAPSVFIFPPSDEQLKSGTASVVCLLNNFYPREAKVQWKVDNALQSGNSQESVTEQDSKDSTYSLSSTLTLSKADYEKHKVYACEVTHQGLSSPVTKSFNRGEC